European Patent Application EP 4 273 247 A1, published November 8, 2023. Title: NUCLEIC ACID, VECTOR AND HOST CELL FOR PREPARING HBV CCCDNA. Applicant: GUANGZHOU EIGHTH PEOPLE'S HOSPITAL, GUANGZHOU MEDICAL UNIVERSITY. Application EP21913020.0. The sequence listing filed with the application follows.

SEQUENCE LISTING (9 sequences)

SEQ ID NO: 1 - DNA, 552 bp, Artificial Sequence
  Core gene
atggacattgacccgtataaagaatttggagcatctgtggagttactctcttttttgccttctgacttctttccttctattcgagatctcctcgacaccgcttctgctctgtatcgggaggccttagagtctccggaacattgttcacctcaccatacagcactcaggcaagctattctgtgttggggtgagttgatgaatctggccacctgggtgggaagtaatttggaagacccagcatccagggaattagtagtcagctatgtcaatgttaatatgggcctaaaaatcagacaactattgtggtttcacatttcctgtcttacttttggaagagaaactgttcttgagtatttggtatcttttggagtgtggattcgcactcctcccgcttacagaccaccaaatgcccctatcttatcaacacttccggaaactactgttgttagacgacgaggcaggtcccctagaagaagaactccctcgcctcgcagacgaagatctcaatcgccgcgtcgcagaagatctcaatctcgggaatctcaatgttag

SEQ ID NO: 2 - DNA, 2532 bp, Artificial Sequence
  Pol gene
atgcccctatcttatcaacacttccggaaactactgttgttagacgacgaggcaggtcccctagaagaagaactccctcgcctcgcagacgaagatctcaatcgccgcgtcgcagaagatctcaatctcgggaatctcaatgttagtatcccttggactcataaggtgggaaactttactgggctttattcttctactgtacctgtctttaatcccgagtggcaaactccctcctttcctcacattcatttacaggaggacattattaatagatgtcaacaatatgtgggccctcttacagttaatgaaaaaaggagattaaaattaattatgcctgctaggttctatcctaaccttaccaaatatttgcccttagacaaaggcattaaaccgtattatcctgaacatgcagttaatcattacttcaaaactaggcattatttacatactctgtggaaggctggcattctatataagagagaaactacacgcagcgcctcattttgtgggtcaccatattcttgggaacaagagctacagcatgggaggttggtcttccaaacctcgacaaggcatggggacgaatctttctgttcccaatcctctgggattctttcccgatcaccagttggaccctgcgttcggagccaactcaaacaatccagattgggacttcaaccccaacaaggatcactggccagaggcaaatcaggtaggagcgggagcattcgggccagggttcaccccaccacacggcggtcttttggggtggagccctcaggctcagggcatattgacaacagtgccagcagcacctcctcctgcctccaccaatcggcagtcaggaagacagcctactcccatctctccacctctaagagacagtcatcctcaggccatgcagtggaactccacaacattccaccaagctctgctagatcccagagtgaggggcctatattttcctgctggtggctccagttccggaacagtaaaccctgttccgactactgcctcacccatatcgtcaatcttctcgaggactggggaccctgcaccgaacatggagaacacaacatcaggattcctaggacccctgctcgtgttacaggcggggtttttcttgttgacaagaatcctcacaataccacagagtctagactcgtggtggacttctctcaattttctagggggagcacccacgtgtcctggccaaaattcgcagtccccaacctccaatcactcaccaacctcttgtcctccaatttgtcctggctatcgctggatgtgtctgcggcgttttatcatattcctcttcatcctgctgctatgcctcatcttcttgttggttcttctggactaccaaggtatgttgcccgtttgtcctctacttccaggaacatcaaccaccagcacggggccatgcaagacctgcacgattcctgctcaaggaacctctatgtttccctcttgttgctgtacaaaaccttcggacggaaactgcacttgtattcccatcccatcatcctgggctttcgcaagattcctatgggagtgggcctcagtccgtttctcctggctcagtttactagtgccatttgttcagtggttcgtagggctttcccccactgtttggctttcagttatatggatgatgtggtattgggggccaagtctgtacaacatcttgagtccctttttacctctattaccaattttcttttgtctttgggtatacatttaaaccctaataaaaccaaacgttggggctactcccttaacttcatgggatatgtaattggaagttggggtactttaccgcaggaacatattgtactaaaactcaagcaatgttttcgaaaattacctgtaaatagacctattgattggaaagtctgtcaaagaattgtgggtcttttgggctttgctgccccttttacacaatgtggctatcctgccttgatgcctttatatgcatgtatacaatctaagcaggctttcactttctcgccaacttacaaggcctttctgtgtaaacaatatctgaacctttaccccgttgcccggcaacggtcaggtctctgccaagtgtttgctgacgcaacccccactggatggggcttggccataggccatcggcgcatgcgtggaacctttgtggctcctctgccgatccatactgcggaactcctagcagcttgtttcgctcgcagccggtctggagcgaaacttatcggcaccgacaactctgttgtcctctctcggaaatacacctcctttccatggctgctagggtgtgctgccaactggatcctgcgcgggacgtcctttgtctacgtcccgtcggcgctgaatcccgcggacgacccgtctcggggccgtttggggctctaccgtccccttcttcatctgccgttccggccgaccacggggcgcacctctctttacgcggtctccccgtctgtgccttctcatctgccggaccgtgtgcacttcgcttcacctctgcacgtcgcatggagaccaccgtga

SEQ ID NO: 3 - DNA, 465 bp, Artificial Sequence
  X gene
atggctgctagggtgtgctgccaactggatcctgcgcgggacgtcctttgtctacgtcccgtcggcgctgaatcccgcggacgacccgtctcggggccgtttggggctctaccgtccccttcttcatctgccgttccggccgaccacggggcgcacctctctttacgcggtctccccgtctgtgccttctcatctgccggaccgtgtgcacttcgcttcacctctgcacgtcgcatggagaccaccgtgaacgcccaccaggtcttgcccaaggtcttacataagaggactcttggactctcagcaatgtcaacgaccgaccttgaggcatacttcaaagactgtgtgtttaaagactgggaggagttgggggaggagattaggttaaaggtctttgtactaggaggctgtaggcataaattggtctgttcaccagcaccatgcaactttttcacctctgcctaa

SEQ ID NO: 4 - DNA, 570 bp, Artificial Sequence
  Reporter gene
atggtgaatggcgtgaaggtgctgtttgccctgatctgcattgctgtggctgaggccaagcccacagagaacaatgaggacttcaacattgtggctgtggcctccaactttgccaccaccgacctggatgccgacaggggcaagctgcctggcaagaagctgcccctggaggtgctgaaggagatggaggccaatgccaggaaggctggctgcaccaggggctgcctgatctgcctgtcccacatcaagtgcacccccaagatgaagaagttcatccctggccggtgccacacctatgagggcgacaaggagtctgcccagggcggcattggcgaggccattgtggacatccctgagatccctggcttcaaggacctggagcccatggagcagttcattgcccaggtggacctgtgtgtggactgcaccaccggctgcctgaagggcctggccaatgtgcagtgctctgacctgctgaagaagtggctgccccagagatgtgccacctttgcctccaaaatccagggccaggtggacaagatcaagggcgctggcggcgatgacacctaa

SEQ ID NO: 5 - DNA, 375 bp, Artificial Sequence
  Antibiotic resistance gene
atggccaagttgaccagtgccgttccggtgctcaccgcgcgcgacgtcgccggagcggtcgagttctggaccgaccggctcgggttctcccgggacttcgtggaggacgacttcgccggtgtggtccgggacgacgtgaccctgttcatcagcgcggtccaggaccaggtggtgccggacaacaccctggcctgggtgtgggtgcgcggcctggacgagctgtacgccgagtggtcggaggtcgtgtccacgaacttccgggacgcctccgggccggccatgaccgagatcggcgagcagccgtgggggcgggagttcgccctgcgcgacccggccggcaactgcgtgcacttcgtggccgaggagcaggactag

SEQ ID NO: 6 - DNA, 4263 bp, Artificial Sequence
  First segment
  misc_feature (2591)..(2591): n is a, c, g, or t
ctgtggaatgtgtgtcagttagggtgtggaaagtccccaggctccccagcaggcagaagtatgcaaagcatgcatctcaattagtcagcaaccaggtgtggaaagtccccaggctccccagcaggcagaagtatgcaaagcatgcatctcaattagtcagcaaccatagtcccgcccctaactccgcccatcccgcccctaactccgcccagttccgcccattctccgccccatggctgactaattttttttatttatgcagaggccgaggccgcctctgcctctgagctattccagaagtagtgaggaggcttttttggaggcctaggcttttgcaaaaagctcccgggagcttgtatatccattttcggatctgatcagcacgtgttgacaattaatcatcggcatagtatatcggcatagtataatacgacagacgcgtctaaaccatggccaagttgaccagtgccgttccggtgctcaccgcgcgcgacgtcgccggagcggtcgagttctggaccgaccggctcgggttctcccgggacttcgtggaggacgacttcgccggtgtggtccgggacgacgtgaccctgttcatcagcgcggtccaggaccaggtggtgccggacaacaccctggcctgggtgtgggtgcgcggcctggacgagctgtacgccgagtggtcggaggtcgtgtccacgaacttccgggacgcctccgggccggccatgaccgagatcggcgagcagccgtgggggcgggagttcgccctgcgcgacccggccggcaactgcgtgcacttcgtggccgaggagcaggacggatccggcgccaccaacttctccctgctgaagcaggctggcgatgtggaggagaaccctgggcccgacattgacccatacaaggagtttggcgcctctgtggagctgctgtccttcctgccatctgacttcttcccatccatcagggacctgctcgacaccgcctctgctctgtatcgggaggccttagagtctccggaacattgttcacctcaccatacagcactcaggcaagccattctgtgttggggtgagttgatgaatctggccacctgggtgggaagtaatttggaagatccagcatccagggaattagtagtcagctatgtcaatgttaatatgggcctaaaaatcagacaactattgtggtttcacatttcctgccttacttttggaagagaaactgttcttgagtatttggtgtcttttggagtgtggattcgcactcctcccgcttacagaccaccaaatgcccctatcttatcaacacttccggaaactactgttgttagatgtcgaggcaggtccactagaagaagaactccctcgcctcgcagacgaagatctcaatcgccgcgtcgcagaagatctcaatctcgggaatctcaatgttagtatcccttggactcataaggtgggaaactttactgggctttattcttctactgtacctatctttaatcctgagtggcaaactccctcctttcctaacattcatttacaggaggacattattaatagatgtcaacaatatgtgggccctcttacagttaatgaaaaaaggagattaaaattaattatgcctgctaggttttatcctaaccttaccaaatatttgcccttggataaaggcattaaaccttattatcctgaacatgcagttaatcattacttcaaaactaggcattatttacatactctgtggaaggctggcattctatataagagagaaactacacgcagcgcttcattttgtgggtcaccatattcttgggaacaagagctacagcatgggaggttggtcttccaaacctcgacaaggcatggggacgaatctttctgttcccaatcctctgggattctttcccgatcaccagttggaccccgcgtttggagccaactcaaacaatccagattgggacttcaaccccaacaaggatcaatggccagaggcaaatcaggtaggagcgggagcattcgggccagggttcaccccaccacacggcggtcttttggggtggagcccccaggctcagggcatattgacaacagtgccagcagctcctcctcctgcctccaccaatcggcagtcaggaagacagcctactcccatctctccacccataagagacagtcatcctcaggccatgcagtggaactccaccacattccaccaagctctgctagatcctgctggtggctccagttccggaacagtaaaccctgttccgactactgcctcacccatatcgtcaatcttctcgaggactggggaccctgcaccgaacatggagagcacaacatcaggattcctaggacccctgctcgtgttacaggcggggtttttcttgttgacaagaatcctcacaataccacagagtctagactcgtggtggacttctctcaattttctagggggagcaccaaagtgtcctggccaaaattcgcagtccccaacctccaatcactcaccaacctcttgtcctccaatttgtcctggctatcgctggatgtgtctgcggcgttttatcatattcctcttcatcctgntgctatgcctcatcttcttgttggttcttctggactaccaaggtatgttgcccgtttgtcctctacttccaggaacatcaaccaccagcacgggaccatgcaagacctgcacgattcctgctcaaggaacctctatgtttccctcttgttgctgtacaaaaccttcggacggaaactgcacttgtattcccatcccatcatcctgggctttcgcaagattcctatgggagtgggcctcagtccgtttctcctggctcagtttactagtgccatttgttcagtggttcgtagggctttcccccactgtttggctttcagttatatggatgatgtggtattgggggccaagtctgtacaacatcttgagtccctttatacctctattaccaattttcttttgtctttgggtatacatttgaaccctaataaaaccaaacgttggggctactcccttaacttcatgggatatgtaattggaagttggggtactttaccacaggaacatattgtactaaaaatcaagcaatgttttcggaaactgcctgtaaatagacctattgattggaaagtgtgtcaaagaattgtgggtcttttgggctttgctgccccttttacacagtgtggctatcctgccttgatgcctttatatgcatgtatacaagctaagcaggctttcactttctcgccaacttacaaggcctttctgtgtaaacaatatctgcacctttaccccgttgcccggcaacggtccggtctctgccaagtgtttgctgacgcaacccccactggatggggcttggccataggccatcggcgcatgcgtggaacctttgtggctcctctgccgatccatactgcggaactcctagcagcttgttttgctcgcagccggtctggagcaaaccttatcgggactgacaactctgttgtcctctctcggaaatacacctccttcccatggctgctcgggtgtgctgccaactggatcctgcgcgggacgtcgtttgtctacgtcccgtcggcgctgaatcccgcggacgacccgtctcggggccgtttgggcctctatcgtccccttcttcatctgccgttccggccgaccacggggcgcacctctctttacgcggtctccccgtctgtgccttctcatctgccggtccgtgtgcacttcgcttcacctctgcacgtcgcatggagaccaccgtgaacgcccaccaggtcttgcccaaggtcttacataagaggactcttggactctcagcaatgtcaacgaccgaccttgaggcatacttcaaagactgtttgtttaaagactgggaggagttgggggaggagaataggttaatgatctttgtactaggaggctgtaggcataaattggtctgtagccccgccccctgtaacttctttactagcgcttaagtttaaacccgctgatcagcctcgactgtgccttctagttgccagccatctgttgtttgcccctcccccgtgccttccttgaccctggaaggtgccactcccactgtcctttcctaataaaatgaggaaattgcatcgcattgtctgagtaggtgtcattctattctggggggtggggtggggcaggacagcaagggggaggattgggaagacaatagcaggcatgcgatcgcgtatacatctccagagg

SEQ ID NO: 7 - DNA, 3449 bp, Artificial Sequence
  Second segment
attaatagtaatcaattacggggtcattagttcatagcccatatatggagttccgcgttacataacttacggtaaatggcccgcctggctgaccgcccaacgacccccgcccattgacgtcaataatgacgtgagttcccatagtaacgccaatagggactttccattgacgtcaatgggaggagtatttacggtaaactgcccacttggcagtacatcaagtgtatcatatgccaagtacgccccctattgacgtcaatgacggtaaatggcccgcctggcattatgcccagtacatgaccttacgggactttcctacttggcagtacatctacgtattagtcatcgctattaccatggtgatgcggttttggcagtacatcaatgggcgtggatagcggtttgactcacggggatttccaagtctccaccccattgacgtcaatgggagtttgttttggcaccaaattcaacgggactttccaaaatgtcgtaataactccgccccattgacgcaaatgggcggtaggcgtgtacgatgggtggtctatataagcgtcgagctccagcaccttgcaactttttcacctctgcctaatcatctcatgttcatgtcctactgttcaagcctccaagctgtgccttgggtggctttggggcctggacattgacccgtataaagaatttggagcttctgtggagttactctcttttttgccttctgacttctttccttctattcgaaccggtatgggtggctcgacgggcagagcgatggtggccaggctagggctggggttgctgcttctggcactgctcctacccacgcagatttactgcaaccaaacatctgttgcaccgtttcccggtaaccagaatatttctgcttccccaaatccaagtaacgctaccaccagagggggtggcagctccctgcagtccacagctggtctcctggctctctctctctctcttctacatctctactgtgtgaatggcgtgaaggtgctgtttgccctgatctgcattgctgtggctgaggccaagcccacagagaacaatgaggacttcaacattgtggctgtggcctccaactttgccaccaccgacctggatgccgacaggggcaagctgcctggcaagaagctgcccctggaggtgctgaaggagatggaggccaatgccaggaaggctggctgcaccaggggctgcctgatctgcctgtcccacatcaagtgcacccccaagatgaagaagttcatccctggccggtgccacacctatgagggcgacaaggagtctgcccagggcggcattggcgaggccattgtggacatccctgagatccctggcttcaaggacctggagcccatggagcagttcattgcccaggtggacctgtgtgtggactgcaccaccggctgcctgaagggcctggccaatgtgcagtgctctgacctgctgaagaagtggctgccccagagatgtgccacctttgcctccaaaatccagggccaggtggacaagatcaagggcgctggcggcgatgacacctaaagtcgacctcgactcttacagttaatgaaaaaaggagattaaaattaattatgcctgctaggttttatcctaaccttaccaaatatttgcccttggataaaggcattaaaccttattatcctgaacatgcagttaatcattacttcaaaactaggcattatttacatactctgtggaaggctggcattctatataagagagaaactacacgcagcgcttcattttgtgggtcaccatattcttgggaacaagagctacagcattcaacaaggcatggggacgaatctttctgttcccaatcctctgggattctttcccgatcaccagttggatcctgcgtttggagccaactcaaacaatccagattgggacttcaaccccaacaaggatcaatggccagaggcaaatcaggtaggagcgggagcattcgggccagggttcaccccaccacacggcggtcttttggggtggagcccccaggctcagggcatattgacaacagtgccagcagctcctcctcctgcctccaccaatcggcagtcaggaagacagcctactcccatctctccacctctaagagacagtcatcctcaggccatgcagtggaactccaccacattccaccaagctctgctagatcctgctggtggctccagttccggaacagtaaaccctgttccgactactgcctcacccatatcgtcaatcttctcgaggactggggaccctgcaccgaacatggagagcacaacatcaggattcctaggacccctgctcgtgttacaggcggggtttttcttgttgacaagaatcctcacaataccacagagtctagaactagtctttacacagtgtggctatcctgccttgatgcctttatatgcatgtatacaagctaagcaggctttcactttctcgccaacttacaaggcctttctgtgtaaacaatatctgcacctttaccccgttgcccggcaacggtccggtctctgccaagtgtttgctgacgcaacccccactggatggggcttggccataggccatcggcgcatgcgtggaacctttgtggctcctctgccgatccatactgcggaactcctagcagcttgttttgctcgcagccggtctggagcaaaccttatcgggactgacaactctgttgtcctctctcggaaatacacctccttcccatggctgctcgggtgtgctgccaactggatcctgcgcgggacgtcgtttgtctacgtcccgtcggcgctgaatcccgcggacgacccgtctcggggccgtttgggcctctatcgtccccttcttcatctgccgttccggccgaccacggggcgcacctctctttacgcggtctccccgtctgtgccttctcatctgccggtccgtgtgcacttcgcttcacctctgcacgtcgcatggagaccaccgtgaacgcccaccaggtcttgcccaaggtcttacataagaggactcttggactctcagcaatgtcaacgaccgaccttgaggcatacttcaaagactgtttgtttaaagactgggaggagttgggggaggagaataggttaaaggtctttgtactaggaggctgtaggcataaattggtctgttcaccagcaccaatgcaactttttcacctctgcctaatcatctcatgttcatgtcctactgttcaagcctccaagctgtgccttgggtggctttagggcatggacattgacccgtataaagaatttggagcttctgtggagttactctcttttttgccttctgacttctttccttctattcgagatctcctcgacaccgcctctgctctgtatcgggaggccttagagtctccggaacattgttcacctcaccatacagcactcaggaattct

SEQ ID NO: 8 - DNA, 30 bp, Artificial Sequence
  Primer 1
cttacataagaggactcttggactctcagc

SEQ ID NO: 9 - DNA, 27 bp, Artificial Sequence
  Primer 2
ggacttcaacattgtggctgtggcctc